European Patent Application EP 4 786 496 A1, published August 5, 2026. Title: 靶向BAFF-R的全人源抗体、CAR-T细胞及其应用. Applicant: 南京驯鹿生物技术股份有限公司. The sequence listing filed with the application follows.

SEQUENCE LISTING (83 sequences)

SEQ ID NO: 1 - DNA, 63 bp, synthetic construct
  source 1..63: mol_type = other DNA; note = Nucleic acid sequence of the CD8alpha signal peptide
atggccctgcctgtgacagctctgctcctccctctggccctgctgctccatgccgccagaccc

SEQ ID NO: 2 - protein, 21 aa, synthetic construct
  source 1..21: note = CD8alpha signal peptide protein sequence
MALPVTALLLPLALLLHAARP

SEQ ID NO: 3 - DNA, 165 bp, synthetic construct
  source 1..165: mol_type = other DNA; note = Nucleic acid sequence of the hinge region of CD8alpha
ttcgtgcccgtgttcctgcccgccaaacctactactacccctgcacctaggcctcccaccccagccccaacaatcgccagccagcctctgtctctgcggcccgaagcctgtagacctgctgccggcggagccgtgcacaccagaggcctggacttcgcctgcgac

SEQ ID NO: 4 - protein, 55 aa, synthetic construct
  source 1..55: note = Protein sequence of the hinge region of CD8alpha
FVPVFLPAKPTTTPAPRPPTPAPTIASQPLSLRPEACRPAAGGAVHTRGLDFACD

SEQ ID NO: 5 - DNA, 84 bp, synthetic construct
  source 1..84: mol_type = other DNA; note = Nucleic acid sequence of the CD8alpha transmembrane region
atctacatctgggcccctctggccggcacctgtggcgtgctgctgctgagcctggtgatcaccctgtactgcaaccaccggaac

SEQ ID NO: 6 - protein, 28 aa, synthetic construct
  source 1..28: note = Protein sequence of the CD8alpha transmembrane region
IYIWAPLAGTCGVLLLSLVITLYCNHRN

SEQ ID NO: 7 - DNA, 126 bp, synthetic construct
  source 1..126: mol_type = other DNA; note = Nucleic acid sequence of the 4-1BB intracellular domain
aaacggggcagaaagaaactcctgtatatattcaaacaaccatttatgagaccagtacaaactactcaagaggaagatggctgtagctgccgatttccagaagaagaagaaggaggatgtgaactg

SEQ ID NO: 8 - protein, 42 aa, synthetic construct
  source 1..42: note = 4-1BB intracellular domain protein sequence
KRGRKKLLYIFKQPFMRPVQTTQEEDGCSCRFPEEEEGGCEL

SEQ ID NO: 9 - DNA, 336 bp, synthetic construct
  source 1..336: mol_type = other DNA; note = Nucleic acid sequence of CD3z intracellular signaling domain
agagtgaagttcagcagatccgccgacgcccctgcctaccagcagggacagaaccagctgtacaacgagctgaacctgggcagacgggaagagtacgacgtgctggacaagcggagaggccgggaccccgagatgggcggaaagcccagacggaagaacccccaggaaggcctgtataacgaactgcagaaagacaagatggccgaggcctacagcgagatcggcatgaagggcgagcggaggcgcggcaagggccacgatggcctgtaccagggcctgagcaccgccaccaaggacacctacgacgccctgcacatgcaggccctgccccccaga

SEQ ID NO: 10 - protein, 112 aa, synthetic construct
  source 1..112: note = CD3z intracellular signaling domain protein sequence
RVKFSRSADAPAYQQGQNQLYNELNLGRREEYDVLDKRRGRDPEMGGKPRRKNPQEGLYNELQKDKMAEAYSEIGMKGERRRGKGHDGLYQGLSTATKDTYDALHMQALPPR

SEQ ID NO: 11 - DNA, 54 bp, synthetic construct
  source 1..54: mol_type = other DNA; note = Cleaved peptide T2A nucleic acid sequence
gagggaaggggcagcttattaacatgtggcgatgtggaagagaaccccggtccc

SEQ ID NO: 12 - protein, 18 aa, synthetic construct
  source 1..18: note = Cleaved peptide T2A protein sequence
EGRGSLLTCGDVEENPGP

SEQ ID NO: 13 - DNA, 66 bp, synthetic construct
  source 1..66: mol_type = other DNA; note = Nucleic acid sequence of CSF2RA signal
atgctgctgctcgtgacctctttactgttatgtgagctgccccaccccgcttttttactgatccct

SEQ ID NO: 14 - protein, 22 aa, synthetic construct
  source 1..22: note = CSF2RA signal protein sequence
MLLLVTSLLLCELPHPAFLLIP

SEQ ID NO: 15 - DNA, 1005 bp, synthetic construct
  source 1..1005: mol_type = other DNA; note = EGFRt nucleic acid sequence
cgtaaggtgtgtaacggaatcggcattggcgagttcaaggactctttaagcatcaacgccacaaacatcaagcacttcaagaattgtacctccatcagcggcgatttacacattctccccgtggcttttcgtggcgattccttcacccacaccccccctctggacccccaagagctggacattttaaaaaccgtgaaggagatcaccggctttctgctgatccaagcttggcccgagaatcgtaccgacctccacgccttcgagaatttagagattattcgtggaaggaccaagcagcacggccagttctctttagccgtcgtgtctttaaacattaccagcctcggtttaaggtctttaaaggagattagcgacggcgacgtgatcatctccggcaacaagaacctctgctacgccaacaccatcaactggaagaagctgttcggaaccagcggccaaaagaccaagatcatcagcaatcgtggagagaactcttgtaaggccactggtcaagtttgccacgccctctgtagccccgaaggatgttggggccccgagcctagggactgtgttagctgcagaaacgtgagcagaggcagagagtgtgtggacaaatgcaatttactggaaggagagcctagggagttcgtggagaacagcgaatgtatccagtgccaccccgagtgtttacctcaagccatgaacatcacttgtaccggaaggggccccgataactgcatccaatgcgcccactacatcgacggaccccactgcgtgaaaacttgtcccgccggagtgatgggagagaataacactttagtgtggaagtacgccgacgctggccacgtctgccatctgtgccaccccaactgtacctacggctgcactggtcccggtttagagggatgtcctaccaacggccccaagatcccctccatcgccaccggaatggtgggcgctctgttattactgctggtggtggctctgggcatcggtttattcatg

SEQ ID NO: 16 - protein, 335 aa, synthetic construct
  source 1..335: note = EGFRt protein sequence
RKVCNGIGIGEFKDSLSINATNIKHFKNCTSISGDLHILPVAFRGDSFTHTPPLDPQELDILKTVKEITGFLLIQAWPENRTDLHAFENLEIIRGRTKQHGQFSLAVVSLNITSLGLRSLKEISDGDVIISGNKNLCYANTINWKKLFGTSGQKTKIISNRGENSCKATGQVCHALCSPEGCWGPEPRDCVSCRNVSRGRECVDKCNLLEGEPREFVENSECIQCHPECLPQAMNITCTGRGPDNCIQCAHYIDGPHCVKTCPAGVMGENNTLVWKYADAGHVCHLCHPNCTYGCTGPGLEGCPTNGPKIPSIATGMVGALLLLLVVALGIGLFM

SEQ ID NO: 17 - DNA, 57 bp, synthetic construct
  source 1..57: mol_type = other DNA; note = The nucleic acid sequence of P2A
gctactaacttcagcctgctgaagcaggctggtgacgtcgaggagaatcctggcccc

SEQ ID NO: 18 - protein, 19 aa, synthetic construct
  source 1..19: note = The protein sequence of P2A
ATNFSLLKQAGDVEENPGP

SEQ ID NO: 19 - DNA, 363 bp, synthetic construct
  source 1..363: mol_type = other DNA; note = BAFF-R-5 CAR VHH nucleic acid sequence
gaggtgcagctggtggagtctgggggaggcgtggtccagcctgggaggtccctgagactcacctgtgcagcctctggattcacgttcagtacctctggcatgtactggattcgccaggctccaggcaaggggctggagtgggtttcatacattagtagtagtagtagtaccatatactacgcagactccgtgaagggccggttcaccatctccagagacaattccaagaacacgctgtatctgcaaatgaacagcctgagagctgaggacacggctgtgtattattgtgtgactcagtcgtgtggtgctggtaaatgctacccgggggtctggggccaagggaccacggtcactgtctcctca

SEQ ID NO: 20 - protein, 121 aa, synthetic construct
  source 1..121: note = Amino acid sequence of BAFF-R-5 CARVHH
EVQLVESGGGVVQPGRSLRLTCAASGFTFSTSGMYWIRQAPGKGLEWVSYISSSSSTIYYADSVKGRFTISRDNSKNTLYLQMNSLRAEDTAVYYCVTQSCGAGKCYPGVWGQGTTVTVSS

SEQ ID NO: 21 - DNA, 741 bp, synthetic construct
  source 1..741: mol_type = other DNA; note = Nucleic acid sequence of Vay736
caggtgcagctgcagcagagcggccccggcctggtgaagcccagccagaccctgagcctgacctgcgccatcagcggcgacagcgtgagcagcaacagcgccgcctggggctggatccgccagagccccggccgcggcctggagtggctgggccgcatctactaccgcagcaagtggtacaacagctacgccgtgagcgtgaagagccgcatcaccatcaaccccgacaccagcaagaaccagttcagcctgcagctgaacagcgtgacccccgaggacaccgccgtgtactactgcgcccgctaccagtgggtgcccaagatcggcgtgttcgacagctggggccagggcaccctggtgaccgtgagcagcggaggaggcggctccggcggcggcggcagcggcggaggaggctctgacatcgtgctgacccagagccccgccaccctgagcctgagccccggcgagcgcgccaccctgagctgccgcgccagccagttcatcctgcccgagtacctgagctggtaccagcagaagcccggccaggccccccgcctgctgatctacggcagcagcagccgcgccaccggcgtgcccgcccgcttcagcggcagcggcagcggcaccgacttcaccctgaccatcagcagcctggagcccgaggacttcgccgtgtactactgccagcagttctacagcagccccctgaccttcggccagggcaccaaggtggagatcaag

SEQ ID NO: 22 - protein, 247 aa, synthetic construct
  source 1..247: note = Amino acid sequence of Vay736
QVQLQQSGPGLVKPSQTLSLTCAISGDSVSSNSAAWGWIRQSPGRGLEWLGRIYYRSKWYNSYAVSVKSRITINPDTSKNQFSLQLNSVTPEDTAVYYCARYQWVPKIGVFDSWGQGTLVTVSSGGGGSGGGGSGGGGSDIVLTQSPATLSLSPGERATLSCRASQFILPEYLSWYQQKPGQAPRLLIYGSSSRATGVPARFSGSGSGTDFTLTISSLEPEDFAVYYCQQFYSSPLTFGQGTKVEIK

SEQ ID NO: 23 - DNA, 732 bp, synthetic construct
  source 1..732: mol_type = other DNA; note = Nucleic acid sequence of city of hope CAR scFV
gtgcagctgcaggagagcggccccggcctggtgaagcccagccagaccctgagccttacttgcacggtgagcggtgacagcatcaccagcggctactggaactggatccgccagcaccccggcaagggcctggagtacatcggctacatcagctacagcggcagcacctactacaaccccagcctgaagagccgcgtgaccatcagccgcgacaccagcaagaaccagtacagcctgaagctgagcagcgtgaccgccgccgacaccgccgtgtactactgcgccagccccaactaccccttctacgccatggactactggggccagggcaccctggtgaccgtgagcagcggcggcggcggcagcggcggcggcggcagcggcggcggcggcagcgacatcgtgctgacccagagccccgccaccctgagcctgagccccggcgagcgcgccaccctgagctgccgcgccagcgagagcgtggacaactacggcatcagcttcatgaactggttccagcagaagcccggccaggccccccgcctgctgatctacgccgccagcaaccgcgccaccggcatccccgcccgcttcagcggcagcggcagcggcaccgacttcaccctgaccatcagcagcctggagcccgaggacttcgccgtgtactactgccagcagagcaaggaggtgccctggaccttcggcggcggcaccaaggtggagatcaagcgc

SEQ ID NO: 24 - protein, 244 aa, synthetic construct
  source 1..244: note = Amino acid sequence of city of hope CAR scFV
VQLQESGPGLVKPSQTLSLTCTVSGDSITSGYWNWIRQHPGKGLEYIGYISYSGSTYYNPSLKSRVTISRDTSKNQYSLKLSSVTAADTAVYYCASPNYPFYAMDYWGQGTLVTVSSGGGGSGGGGSGGGGSDIVLTQSPATLSLSPGERATLSCRASESVDNYGISFMNWFQQKPGQAPRLLIYAASNRATGIPARFSGSGSGTDFTLTISSLEPEDFAVYYCQQSKEVPWTFGGGTKVEIKR

SEQ ID NO: 25 - protein, 121 aa, synthetic construct; identical to SEQ ID NO: 20
  source 1..121: note = The amino acid sequence of 05VH

SEQ ID NO: 26 - DNA, 363 bp, synthetic construct; identical to SEQ ID NO: 19
  source 1..363: mol_type = other DNA; note = The nucleotide sequence of 05VH

SEQ ID NO: 27 - protein, 8 aa, synthetic construct
  source 1..8: note = 05VH CDR1
GFTFSTSG

SEQ ID NO: 28 - protein, 8 aa, synthetic construct
  source 1..8: note = 05VH CDR2
ISSSSSTI

SEQ ID NO: 29 - protein, 14 aa, synthetic construct
  source 1..14: note = 05VH CDR3
VTQSCGAGKCYPGV

SEQ ID NO: 30 - protein, 108 aa, synthetic construct
  source 1..108: note = Amino acid sequence of 01VL
DIQMTQSPSSLSASVGDRVTITCRASQKISSYLNWYQQKPGKAPKLLIYAASSLQSGVPSRFSGSGSGADFTLTISSLQPEDFATYYCQQSYSPPTTFGGGTKVDIKR

SEQ ID NO: 31 - DNA, 324 bp, synthetic construct
  source 1..324: mol_type = other DNA; note = Nucleotide sequence of 01VL
gacatccagatgacccagtctccatcctccctgtctgcatctgttggagacagagtcaccatcacttgccgggcaagtcagaaaattagcagctatttaaattggtatcagcagaaaccagggaaagcccctaagctcctgatctatgctgcatccagtttgcaaagtggggtcccatcaaggttcagtggcagtggatctggggcagatttcactctcaccatcagcagtctgcaacctgaagattttgcaacttactactgtcagcagagttacagtcccccgaccactttcggcggagggaccaaagtggatatcaaacgt

SEQ ID NO: 32 - protein, 128 aa, synthetic construct
  source 1..128: note = Amino acid sequence of 01VH
MAEVQLVESGAEVKKPGASVKVSCKASGYTFTSYGISWVRQAPGQGLEWMGWISAYNGNTNYAQKLQGRVTMTTDTSTSTAYMELRSLRSDDTAVYYCARNTYYYDSSGYPNDAFDIWGQGTTVTVSS

SEQ ID NO: 33 - DNA, 384 bp, synthetic construct
  source 1..384: mol_type = other DNA; note = 01VH nucleotide sequence
atggccgaggtgcagctggtggagtctggagctgaggtgaagaagcctggggcctcagtgaaggtctcctgcaaggcttctggttacacctttaccagctatggtatcagctgggtgcgacaggcccctggacaagggcttgagtggatgggatggatcagcgcttacaatggtaacacaaactatgcacagaagctccagggcagagtcaccatgaccacagacacatccacgagcacagcctacatggagctgaggagcctgagatctgacgacacggccgtgtattactgtgcgagaaatacgtattactatgatagtagtggttacccaaatgatgcttttgatatctggggccaagggaccacggtcaccgtctcctca

SEQ ID NO: 34 - protein, 255 aa, synthetic construct
  source 1..255: note = Amino acid sequence of the scFv(VL-VH) contained in the CAR constructed from clone 1 (01)
DIQMTQSPSSLSASVGDRVTITCRASQKISSYLNWYQQKPGKAPKLLIYAASSLQSGVPSRFSGSGSGADFTLTISSLQPEDFATYYCQQSYSPPTTFGGGTKVDIKRSRGGGGSGGGGSGGGGSLEMAEVQLVESGAEVKKPGASVKVSCKASGYTFTSYGISWVRQAPGQGLEWMGWISAYNGNTNYAQKLQGRVTMTTDTSTSTAYMELRSLRSDDTAVYYCARNTYYYDSSGYPNDAFDIWGQGTTVTVSS

SEQ ID NO: 35 - DNA, 765 bp, synthetic construct
  source 1..765: mol_type = other DNA; note = Nucleotide sequence of the scFv(VL-VH) contained in the CAR constructed from clone 1 (01)
gacatccagatgacccagtctccatcctccctgtctgcatctgttggagacagagtcaccatcacttgccgggcaagtcagaaaattagcagctatttaaattggtatcagcagaaaccagggaaagcccctaagctcctgatctatgctgcatccagtttgcaaagtggggtcccatcaaggttcagtggcagtggatctggggcagatttcactctcaccatcagcagtctgcaacctgaagattttgcaacttactactgtcagcagagttacagtcccccgaccactttcggcggagggaccaaagtggatatcaaacgttctagaggtggtggtggtagcggcggcggcggctctggtggtggtggatccctcgagatggccgaggtgcagctggtggagtctggagctgaggtgaagaagcctggggcctcagtgaaggtctcctgcaaggcttctggttacacctttaccagctatggtatcagctgggtgcgacaggcccctggacaagggcttgagtggatgggatggatcagcgcttacaatggtaacacaaactatgcacagaagctccagggcagagtcaccatgaccacagacacatccacgagcacagcctacatggagctgaggagcctgagatctgacgacacggccgtgtattactgtgcgagaaatacgtattactatgatagtagtggttacccaaatgatgcttttgatatctggggccaagggaccacggtcaccgtctcctca

SEQ ID NO: 36 - protein, 6 aa, synthetic construct
  source 1..6: note = 01VL CDR1
QKISSY

SEQ ID NO: 37 - protein, 9 aa, synthetic construct
  source 1..9: note = 01VL CDR3
QQSYSPPTT

SEQ ID NO: 38 - protein, 8 aa, synthetic construct
  source 1..8: note = 01VH CDR1
GYTFTSYG

SEQ ID NO: 39 - protein, 8 aa, synthetic construct
  source 1..8: note = 01VH CDR2
ISAYNGNT

SEQ ID NO: 40 - protein, 19 aa, synthetic construct
  source 1..19: note = 01VH CDR3
ARNTYYYDSSGYPNDAFDI

SEQ ID NO: 41 - protein, 229 aa, synthetic construct
  source 1..229: note = hFc PAA Hs
ESKYGPPCPPCPAPEAAGGPSVFLFPPKPKDTLMISRTPEVTCVVVDVSQEDPEVQFNWYVDGVEVHNAKTKPREEQFNSTYRVVSVLTVLHQDWLNGKEYKCKVSNKGLPSSIEKTISKAKGQPREPQVCTLPPSQEEMTKNQVSLSCAVKGFYPSDIAVEWESNGQPENNYKTTPPVLDSDGSFFLVSRLTVDKSRWQEGNVFSCSVMHEALHNHYTQKSLSLSLGK

SEQ ID NO: 42 - DNA, 687 bp, synthetic construct
  source 1..687: mol_type = other DNA; note = Nucleotide sequence of hFc PAA Hs
gagagcaagtacggccccccctgccccccctgccccgcccccgaggccgccggcggccccagcgtgttcctgttcccccccaagcccaaggacaccctgatgatcagccgcacccccgaggtgacctgcgtggtggtggacgtgagccaggaggaccccgaggtgcagttcaactggtacgtggacggcgtggaggtgcacaacgccaagaccaagccccgcgaggagcagttcaacagcacctaccgcgtggtgagcgtgctgaccgtgctgcaccaggactggctgaacggcaaggagtacaagtgcaaggtgagcaacaagggcctgcccagcagcatcgagaagaccatcagcaaggccaagggccagccccgcgagccccaggtgtgcaccctgccccccagccaggaggagatgaccaagaaccaggtgagcctgagctgcgccgtgaagggcttctaccccagcgacatcgccgtggagtgggagagcaacggccagcccgagaacaactacaagaccaccccccccgtgctggacagcgacggcagcttcttcctggtgagcagactgaccgtggacaagagccgctggcaggagggcaacgtgttcagctgcagcgtgatgcacgaggccctgcacaaccactacacccagaagagcctgagcctgagcctgggcaag

SEQ ID NO: 43 - protein, 229 aa, synthetic construct
  source 1..229: note = Nucleotide sequence of hFc PAA Ks
ESKYGPPCPPCPAPEAAGGPSVFLFPPKPKDTLMISRTPEVTCVVVDVSQEDPEVQFNWYVDGVEVHNAKTKPREEQFNSTYRVVSVLTVLHQDWLNGKEYKCKVSNKGLPSSIEKTISKAKGQPREPQVYTLPPCQEEMTKNQVSLWCLVKGFYPSDIAVEWESNGQPENNYKTTPPVLDSDGSFFLYSRLTVDKSRWQEGNVFSCSVMHEALHNHYTQKSLSLSLGK

SEQ ID NO: 44 - DNA, 687 bp, synthetic construct
  source 1..687: mol_type = other DNA; note = hFc PAA Ks
gagagcaagtacggccccccctgccccccctgccccgcccccgaggccgccggcggccccagcgtgttcctgttcccccccaagcccaaggacaccctgatgatcagccgcacccccgaggtgacctgcgtggtggtggacgtgagccaggaggaccccgaggtgcagttcaactggtacgtggacggcgtggaggtgcacaacgccaagaccaagccccgcgaggagcagttcaacagcacctaccgcgtggtgagcgtgctgaccgtgctgcaccaggactggctgaacggcaaggagtacaagtgcaaggtgagcaacaagggcctgcccagcagcatcgagaagaccatcagcaaggccaagggccagccccgcgagccccaggtgtacaccctgcccccctgccaggaggagatgaccaagaaccaggtgagcctgtggtgcctggtgaagggcttctaccccagcgacatcgccgtggagtgggagagcaacggccagcccgagaacaactacaagaccaccccccccgtgctggacagcgacggcagcttcttcctgtacagcagactgaccgtggacaagagccgctggcaggagggcaacgtgttcagctgcagcgtgatgcacgaggccctgcacaaccactacacccagaagagcctgagcctgagcctgggcaag

SEQ ID NO: 45 - protein, 119 aa, synthetic construct
  source 1..119: note = OKT3 VH
QVQLVQSGGGVVQPGRSLRLSCKASGYTFTRYTMHWVRQAPGKGLEWIGYINPSRGYTNYNQKFKDRFTISRDNSKNTAFLQMDSLRPEDTGVYFCARYYDDHYCLDYWGQGTPVTVSS

SEQ ID NO: 46 - DNA, 357 bp, synthetic construct
  source 1..357: mol_type = other DNA; note = Nucleotide sequence of OKT3 VH
caggtgcagctggtgcagagcggcggcggcgtggtgcagcccggccgcagcctgcgcctgagctgcaaggccagcggctacaccttcacccgctacaccatgcactgggtgcgccaggcccccggcaagggcctggagtggatcggctacatcaaccccagccgcggctacaccaactacaaccagaagttcaaggaccgcttcaccatcagccgcgacaacagcaagaacaccgccttcctgcagatggacagcctgcgccccgaggacaccggcgtgtacttctgcgcccgctactacgacgaccactactgcctggactactggggccagggcacccccgtgaccgtgagcagc

SEQ ID NO: 47 - protein, 107 aa, synthetic construct
  source 1..107: note = OKT3 VK
DIQMTQSPSSLSASVGDRVTITCSASSSVSYMNWYQQTPGKAPKRWIYDTSKLASGVPSRFSGSGSGTDYTFTISSLQPEDIATYYCQQWSSNPFTFGQGTKLQITR

SEQ ID NO: 48 - DNA, 321 bp, synthetic construct
  source 1..321: mol_type = other DNA; note = Nucleotide sequence of OKT3 VK
gacatccagatgacccagagccccagcagcctgagcgccagcgtgggcgaccgcgtgaccatcacctgcagcgccagcagcagcgtgagctacatgaactggtaccagcagacccccggcaaggcccccaagcgctggatctacgacaccagcaagctggccagcggcgtgcccagccgcttcagcggcagcggcagcggcaccgactacaccttcaccatcagcagcctgcagcccgaggacatcgccacctactactgccagcagtggagcagcaaccccttcaccttcggccagggcaccaagctgcagatcacccgc

SEQ ID NO: 49 - protein, 461 aa, synthetic construct
  source 1..461: note = OKT3 scFab
DIQMTQSPSSLSASVGDRVTITCSASSSVSYMNWYQQTPGKAPKRWIYDTSKLASGVPSRFSGSGSGTDYTFTISSLQPEDIATYYCQQWSSNPFTFGQGTKLQITRRTVAAPSVFIFPPSDEQLKSGTASVVCLLNNFYPREAKVQWKVDNALQSGNSQESVTEQDSKDSTYSLSSTLTLSKADYEKHKVYACEVTHQGLSSPVTKSFNRGECGGGGSGGGGSGGGGSGGGGSGGGGSGGGGSQVQLVQSGGGVVQPGRSLRLSCKASGYTFTRYTMHWVRQAPGKGLEWIGYINPSRGYTNYNQKFKDRFTISRDNSKNTAFLQMDSLRPEDTGVYFCARYYDDHYCLDYWGQGTPVTVSSASTKGPSVFPLAPCSRSTSESTAALGCLVKDYFPEPVTVSWNSGALTSGVHTFPAVLQSSGLYSLSSVVTVPSSSLGTKTYTCNVDHKPSNTKVDKRV

SEQ ID NO: 50 - DNA, 1383 bp, synthetic construct
  source 1..1383: mol_type = other DNA; note = Nucleotide sequence of the OKT3 scFab
gacatccagatgacccagagccccagcagcctgagcgccagcgtgggcgaccgcgtgaccatcacctgcagcgccagcagcagcgtgagctacatgaactggtaccagcagacccccggcaaggcccccaagcgctggatctacgacaccagcaagctggccagcggcgtgcccagccgcttcagcggcagcggcagcggcaccgactacaccttcaccatcagcagcctgcagcccgaggacatcgccacctactactgccagcagtggagcagcaaccccttcaccttcggccagggcaccaagctgcagatcacccgccgtacggtggccgcaccaagcgtcttcatcttcccgccatctgatgagcagttgaaatctggaactgcctctgttgtgtgcctgctgaataacttctatcccagagaggccaaagtacagtggaaggtggataacgccctccaatcgggtaactcccaggagagtgtcacagagcaggacagcaaggacagcacctacagcctcagcagcaccctgacgctgagcaaagcagactacgagaaacacaaagtctacgcctgcgaagtcacccatcagggcctgagctcgcccgtcacaaagagctttaacagaggcgagtgcggcggcggcggatccggcggcggcggaagcggcggcggcggatccggcggcggcggaagcggcggcggcggatccggcggcggaggaagccaggtgcagctggtgcagagcggcggcggcgtggtgcagcccggccgcagcctgcgcctgagctgcaaggccagcggctacaccttcacccgctacaccatgcactgggtgcgccaggcccccggcaagggcctggagtggatcggctacatcaaccccagccgcggctacaccaactacaaccagaagttcaaggaccgcttcaccatcagccgcgacaacagcaagaacaccgccttcctgcagatggacagcctgcgccccgaggacaccggcgtgtacttctgcgcccgctactacgacgaccactactgcctggactactggggccagggcacccccgtgaccgtgagcagcgctagcaccaagggccccagcgtgttccccctggccccctgcagccgcagcaccagcgagagcaccgccgccctgggctgcctggtgaaggactacttccccgagcccgtgaccgtgagctggaacagcggcgccctgaccagcggcgtgcacaccttccccgccgtgctgcagagcagcggcctgtacagcctgagcagcgtggtgaccgtgcccagcagcagcctgggcaccaagacctacacctgcaacgtggaccacaagcccagcaacaccaaggtggacaagcgcgtg

SEQ ID NO: 51 - protein, 350 aa, synthetic construct
  source 1..350: note = 05VH-hFc PAA Hs
EVQLVESGGGVVQPGRSLRLTCAASGFTFSTSGMYWIRQAPGKGLEWVSYISSSSSTIYYADSVKGRFTISRDNSKNTLYLQMNSLRAEDTAVYYCVTQSCGAGKCYPGVWGQGTTVTVSSESKYGPPCPPCPAPEAAGGPSVFLFPPKPKDTLMISRTPEVTCVVVDVSQEDPEVQFNWYVDGVEVHNAKTKPREEQFNSTYRVVSVLTVLHQDWLNGKEYKCKVSNKGLPSSIEKTISKAKGQPREPQVCTLPPSQEEMTKNQVSLSCAVKGFYPSDIAVEWESNGQPENNYKTTPPVLDSDGSFFLVSRLTVDKSRWQEGNVFSCSVMHEALHNHYTQKSLSLSLGK

SEQ ID NO: 52 - protein, 1050 aa, synthetic construct
  source 1..1050: note = Nucleotide sequence of the 05VH-hFc PAA Hs
GAGGTGCAGCTGGTGGAGTCTGGGGGAGGCGTGGTCCAGCCTGGGAGGTCCCTGAGACTCACCTGTGCAGCCTCTGGATTCACGTTCAGTACCTCTGGCATGTACTGGATTCGCCAGGCTCCAGGCAAGGGGCTGGAGTGGGTTTCATACATTAGTAGTAGTAGTAGTACCATATACTACGCAGACTCCGTGAAGGGCCGGTTCACCATCTCCAGAGACAATTCCAAGAACACGCTGTATCTGCAAATGAACAGCCTGAGAGCTGAGGACACGGCTGTGTATTATTGTGTGACTCAGTCGTGTGGTGCTGGTAAATGCTACCCGGGGGTCTGGGGCCAAGGGACCACGGTCACTGTCTCCTCAGAGAGCAAGTACGGCCCCCCCTGCCCCCCCTGCCCCGCCCCCGAGGCCGCCGGCGGCCCCAGCGTGTTCCTGTTCCCCCCCAAGCCCAAGGACACCCTGATGATCAGCCGCACCCCCGAGGTGACCTGCGTGGTGGTGGACGTGAGCCAGGAGGACCCCGAGGTGCAGTTCAACTGGTACGTGGACGGCGTGGAGGTGCACAACGCCAAGACCAAGCCCCGCGAGGAGCAGTTCAACAGCACCTACCGCGTGGTGAGCGTGCTGACCGTGCTGCACCAGGACTGGCTGAACGGCAAGGAGTACAAGTGCAAGGTGAGCAACAAGGGCCTGCCCAGCAGCATCGAGAAGACCATCAGCAAGGCCAAGGGCCAGCCCCGCGAGCCCCAGGTGTGCACCCTGCCCCCCAGCCAGGAGGAGATGACCAAGAACCAGGTGAGCCTGAGCTGCGCCGTGAAGGGCTTCTACCCCAGCGACATCGCCGTGGAGTGGGAGAGCAACGGCCAGCCCGAGAACAACTACAAGACCACCCCCCCCGTGCTGGACAGCGACGGCAGCTTCTTCCTGGTGAGCAGACTGACCGTGGACAAGAGCCGCTGGCAGGAGGGCAACGTGTTCAGCTGCAGCGTGATGCACGAGGCCCTGCACAACCACTACACCCAGAAGAGCCTGAGCCTGAGCCTGGGCAAG

SEQ ID NO: 53 - protein, 690 aa, synthetic construct
  source 1..690: note = OKT3 scFab-H PAA Ks
DIQMTQSPSSLSASVGDRVTITCSASSSVSYMNWYQQTPGKAPKRWIYDTSKLASGVPSRFSGSGSGTDYTFTISSLQPEDIATYYCQQWSSNPFTFGQGTKLQITRRTVAAPSVFIFPPSDEQLKSGTASVVCLLNNFYPREAKVQWKVDNALQSGNSQESVTEQDSKDSTYSLSSTLTLSKADYEKHKVYACEVTHQGLSSPVTKSFNRGECGGGGSGGGGSGGGGSGGGGSGGGGSGGGGSQVQLVQSGGGVVQPGRSLRLSCKASGYTFTRYTMHWVRQAPGKGLEWIGYINPSRGYTNYNQKFKDRFTISRDNSKNTAFLQMDSLRPEDTGVYFCARYYDDHYCLDYWGQGTPVTVSSASTKGPSVFPLAPCSRSTSESTAALGCLVKDYFPEPVTVSWNSGALTSGVHTFPAVLQSSGLYSLSSVVTVPSSSLGTKTYTCNVDHKPSNTKVDKRVESKYGPPCPPCPAPEAAGGPSVFLFPPKPKDTLMISRTPEVTCVVVDVSQEDPEVQFNWYVDGVEVHNAKTKPREEQFNSTYRVVSVLTVLHQDWLNGKEYKCKVSNKGLPSSIEKTISKAKGQPREPQVYTLPPCQEEMTKNQVSLWCLVKGFYPSDIAVEWESNGQPENNYKTTPPVLDSDGSFFLYSRLTVDKSRWQEGNVFSCSVMHEALHNHYTQKSLSLSLGK

SEQ ID NO: 54 - DNA, 2070 bp, synthetic construct
  source 1..2070: mol_type = other DNA; note = Nucleotide sequence of OKT3 scFab-H PAA Ks
gacatccagatgacccagagccccagcagcctgagcgccagcgtgggcgaccgcgtgaccatcacctgcagcgccagcagcagcgtgagctacatgaactggtaccagcagacccccggcaaggcccccaagcgctggatctacgacaccagcaagctggccagcggcgtgcccagccgcttcagcggcagcggcagcggcaccgactacaccttcaccatcagcagcctgcagcccgaggacatcgccacctactactgccagcagtggagcagcaaccccttcaccttcggccagggcaccaagctgcagatcacccgccgtacggtggccgcaccaagcgtcttcatcttcccgccatctgatgagcagttgaaatctggaactgcctctgttgtgtgcctgctgaataacttctatcccagagaggccaaagtacagtggaaggtggataacgccctccaatcgggtaactcccaggagagtgtcacagagcaggacagcaaggacagcacctacagcctcagcagcaccctgacgctgagcaaagcagactacgagaaacacaaagtctacgcctgcgaagtcacccatcagggcctgagctcgcccgtcacaaagagctttaacagaggcgagtgcggcggcggcggatccggcggcggcggaagcggcggcggcggatccggcggcggcggaagcggcggcggcggatccggcggcggaggaagccaggtgcagctggtgcagagcggcggcggcgtggtgcagcccggccgcagcctgcgcctgagctgcaaggccagcggctacaccttcacccgctacaccatgcactgggtgcgccaggcccccggcaagggcctggagtggatcggctacatcaaccccagccgcggctacaccaactacaaccagaagttcaaggaccgcttcaccatcagccgcgacaacagcaagaacaccgccttcctgcagatggacagcctgcgccccgaggacaccggcgtgtacttctgcgcccgctactacgacgaccactactgcctggactactggggccagggcacccccgtgaccgtgagcagcgctagcaccaagggccccagcgtgttccccctggccccctgcagccgcagcaccagcgagagcaccgccgccctgggctgcctggtgaaggactacttccccgagcccgtgaccgtgagctggaacagcggcgccctgaccagcggcgtgcacaccttccccgccgtgctgcagagcagcggcctgtacagcctgagcagcgtggtgaccgtgcccagcagcagcctgggcaccaagacctacacctgcaacgtggaccacaagcccagcaacaccaaggtggacaagcgcgtggagagcaagtacggccccccctgccccccctgccccgcccccgaggccgccggcggccccagcgtgttcctgttcccccccaagcccaaggacaccctgatgatcagccgcacccccgaggtgacctgcgtggtggtggacgtgagccaggaggaccccgaggtgcagttcaactggtacgtggacggcgtggaggtgcacaacgccaagaccaagccccgcgaggagcagttcaacagcacctaccgcgtggtgagcgtgctgaccgtgctgcaccaggactggctgaacggcaaggagtacaagtgcaaggtgagcaacaagggcctgcccagcagcatcgagaagaccatcagcaaggccaagggccagccccgcgagccccaggtgtacaccctgcccccctgccaggaggagatgaccaagaaccaggtgagcctgtggtgcctggtgaagggcttctaccccagcgacatcgccgtggagtgggagagcaacggccagcccgagaacaactacaagaccaccccccccgtgctggacagcgacggcagcttcttcctgtacagcagactgaccgtggacaagagccgctggcaggagggcaacgtgttcagctgcagcgtgatgcacgaggccctgcacaaccactacacccagaagagcctgagcctgagcctgggcaag

SEQ ID NO: 55 - protein, 229 aa, synthetic construct
  source 1..229: note = hFc PE
ESKYGPPCPPCPAPEFEGGPSVFLFPPKPKDTLMISRTPEVTCVVVDVSQEDPEVQFNWYVDGVEVHNAKTKPREEQFNSTYRVVSVLTVLHQDWLNGKEYKCKVSNKGLPSSIEKTISKAKGQPREPQVYTLPPSQEEMTKNQVSLTCLVKGFYPSDIAVEWESNGQPENNYKTTPPVLDSDGSFFLYSRLTVDKSRWQEGNVFSCSVMHEALHNHYTQKSLSLSLGK

SEQ ID NO: 56 - protein, 687 aa, synthetic construct
  source 1..687: note = Nucleotide sequence of hFc PE
GAGAGCAAGTACGGCCCTCCCTGCCCACCCTGCCCCGCTCCCGAGTTTGAAGGCGGCCCCAGCGTGTTCCTGTTCCCCCCCAAGCCCAAGGACACCCTGATGATCAGCCGCACCCCCGAGGTGACCTGCGTGGTGGTGGACGTGAGCCAGGAGGACCCCGAGGTGCAGTTCAACTGGTACGTGGACGGCGTGGAGGTGCACAACGCCAAGACCAAGCCCCGCGAGGAGCAGTTCAACAGCACCTACCGCGTGGTGAGCGTGCTGACCGTGCTGCACCAGGACTGGCTGAACGGCAAGGAGTACAAGTGCAAGGTGAGCAACAAGGGCCTGCCCAGCAGCATCGAGAAGACCATCAGCAAGGCCAAGGGCCAGCCCCGCGAGCCCCAGGTGTACACCCTGCCCCCCAGCCAGGAGGAGATGACCAAGAACCAGGTGAGCCTGACCTGCCTGGTGAAGGGCTTCTACCCCAGCGACATCGCCGTGGAGTGGGAGAGCAACGGCCAGCCCGAGAACAACTACAAGACCACCCCCCCCGTGCTGGACAGCGACGGCAGCTTCTTCCTGTACAGCAGACTGACCGTGGACAAGAGCCGCTGGCAGGAGGGCAACGTGTTCAGCTGCAGCGTGATGCACGAGGCCCTGCACAACCACTACACCCAGAAGAGCCTGAGCCTGAGCCTGGGCAAG

SEQ ID NO: 57 - protein, 350 aa, synthetic construct
  source 1..350: note = 05VH-hFc PE
EVQLVESGGGVVQPGRSLRLTCAASGFTFSTSGMYWIRQAPGKGLEWVSYISSSSSTIYYADSVKGRFTISRDNSKNTLYLQMNSLRAEDTAVYYCVTQSCGAGKCYPGVWGQGTTVTVSSESKYGPPCPPCPAPEFEGGPSVFLFPPKPKDTLMISRTPEVTCVVVDVSQEDPEVQFNWYVDGVEVHNAKTKPREEQFNSTYRVVSVLTVLHQDWLNGKEYKCKVSNKGLPSSIEKTISKAKGQPREPQVYTLPPSQEEMTKNQVSLTCLVKGFYPSDIAVEWESNGQPENNYKTTPPVLDSDGSFFLYSRLTVDKSRWQEGNVFSCSVMHEALHNHYTQKSLSLSLGK

SEQ ID NO: 58 - protein, 1050 aa, synthetic construct
  source 1..1050: note = 05 VH-hFC PE nucleotide sequence
GAGGTGCAGCTGGTGGAGTCTGGGGGAGGCGTGGTCCAGCCTGGGAGGTCCCTGAGACTCACCTGTGCAGCCTCTGGATTCACGTTCAGTACCTCTGGCATGTACTGGATTCGCCAGGCTCCAGGCAAGGGGCTGGAGTGGGTTTCATACATTAGTAGTAGTAGTAGTACCATATACTACGCAGACTCCGTGAAGGGCCGGTTCACCATCTCCAGAGACAATTCCAAGAACACGCTGTATCTGCAAATGAACAGCCTGAGAGCTGAGGACACGGCTGTGTATTATTGTGTGACTCAGTCGTGTGGTGCTGGTAAATGCTACCCGGGGGTCTGGGGCCAAGGGACCACGGTCACTGTCTCCTCAGAGAGCAAGTACGGCCCTCCCTGCCCACCCTGCCCCGCTCCCGAGTTTGAAGGCGGCCCCAGCGTGTTCCTGTTCCCCCCCAAGCCCAAGGACACCCTGATGATCAGCCGCACCCCCGAGGTGACCTGCGTGGTGGTGGACGTGAGCCAGGAGGACCCCGAGGTGCAGTTCAACTGGTACGTGGACGGCGTGGAGGTGCACAACGCCAAGACCAAGCCCCGCGAGGAGCAGTTCAACAGCACCTACCGCGTGGTGAGCGTGCTGACCGTGCTGCACCAGGACTGGCTGAACGGCAAGGAGTACAAGTGCAAGGTGAGCAACAAGGGCCTGCCCAGCAGCATCGAGAAGACCATCAGCAAGGCCAAGGGCCAGCCCCGCGAGCCCCAGGTGTACACCCTGCCCCCCAGCCAGGAGGAGATGACCAAGAACCAGGTGAGCCTGACCTGCCTGGTGAAGGGCTTCTACCCCAGCGACATCGCCGTGGAGTGGGAGAGCAACGGCCAGCCCGAGAACAACTACAAGACCACCCCCCCCGTGCTGGACAGCGACGGCAGCTTCTTCCTGTACAGCAGACTGACCGTGGACAAGAGCCGCTGGCAGGAGGGCAACGTGTTCAGCTGCAGCGTGATGCACGAGGCCCTGCACAACCACTACACCCAGAAGAGCCTGAGCCTGAGCCTGGGCAAG

SEQ ID NO: 59 - protein, 184 aa, synthetic construct
  source 1..184: note = human BAFF-R
MRRGPRSLRGRDAPAPTPCVPAECFDLLVRHCVACGLLRTPRPKPAGASSPAPRTALQPQESVGAGAGEAALPLPGLLFGAPALLGLALVLALVLVGLVSWRRRQRRLRGASSAEAPDGDKDAPEPLDKVIILSPGISDATAPAWPPPGEDPGTTPPGHSVPVPATELGSTELVTTKTAGPEQQ

SEQ ID NO: 60 - protein, 184 aa, synthetic construct
  source 1..184: note = cynomolgus BAFF-R
MKRGPRSLRGRDAPAPTPCVPAECFDLLVRHCVACGLLRTPRPKPAPASSPAPRTALQPQESVGAGAGEAALSLPGLLFGAPALLGLALVLALVLVGLVSWRRRQRRLRGASSAEAPDGDKDKDEPLDKVIILSPGISDAAAPAWPPPGEDPGTTPPGHSVPVPATELGSTELVTTKTAGPEQQ

SEQ ID NO: 61 - protein, 175 aa, synthetic construct
  source 1..175: note = mouse BAFF-R
MGARRLRVRSQRSRDSSVPTQCNQTECFDPLVRNCVSCELFHTPDTGHTSSLEPGTALQPQEGSALRPDVALLVGAPALLGLILALTLVGLVSLVSWRWRQQLRTASPDTSEGVQQESLENVFVPSSETPHASAPTWPPLKEDADSALPRHSVPVPATELGSTELVTTKTAGPEQ

SEQ ID NO: 62 - protein, 78 aa, synthetic construct
  source 1..78: note = Extracellular domain of human BAFF-R
MRRGPRSLRGRDAPAPTPCVPAECFDLLVRHCVACGLLRTPRPKPAGASSPAPRTALQPQESVGAGAGEAALPLPGLL

SEQ ID NO: 63 - protein, 78 aa, synthetic construct
  source 1..78: note = cynomolgus BAFF-R extracellular region
MKRGPRSLRGRDAPAPTPCVPAECFDLLVRHCVACGLLRTPRPKPAPASSPAPRTALQPQESVGAGAGEAALSLPGLL

SEQ ID NO: 64 - protein, 73 aa, synthetic construct
  source 1..73: note = mouse BAFF-R extracellular domain
MGARRLRVRSQRSRDSSVPTQCNQTECFDPLVRNCVSCELFHTPDTGHTSSLEPGTALQPQEGSALRPDVALL

SEQ ID NO: 65 - protein, 125 aa, synthetic construct
  source 1..125: note = SP34 VH
EVQLVESGGGLVQPKGSLKLSCAASGFTFNTYAMNWVRQAPGKGLEWVARIRSKYNNYATYYADSVKDRFTISRDDSQSILYLQMNNLKTEDTAMYYCVRHGNFGNSYVSWFAYWGQGTLVTVSS

SEQ ID NO: 66 - DNA, 375 bp, synthetic construct
  source 1..375: mol_type = other DNA; note = Nucleotide sequence of SP34 VH
gaggtgcagctggtggagagcggcggcggcctggtgcagcccaagggcagcctgaagctgagctgcgccgccagcggcttcaccttcaacacctacgccatgaactgggtgcgccaggcccccggcaagggcctggagtgggtggcccgcatccgcagcaagtacaacaactacgccacctactacgccgacagcgtgaaggaccgcttcaccatcagccgcgacgacagccagagcatcctgtacctgcagatgaacaacctgaagaccgaggacaccgccatgtactactgcgtgcgccacggcaacttcggcaacagctacgtgagctggttcgcctactggggccagggcaccctggtgaccgtgagcagc

SEQ ID NO: 67 - protein, 109 aa, synthetic construct
  source 1..109: note = SP34 VL
QAVVTQESALTTSPGETVTLTCRSSTGAVTTSNYANWVQEKPDHLFTGLIGGTNKRAPGVPARFSGSLIGDKAALTITGAQTEDEAIYFCALWYSNLWVFGGGTKLTVL

SEQ ID NO: 68 - DNA, 327 bp, synthetic construct
  source 1..327: mol_type = other DNA; note = Nucleotide sequence of the SP34 VL
caggccgtggtgacccaggagagcgccctgaccaccagccccggcgagaccgtgaccctgacctgccgcagcagcaccggcgccgtgaccaccagcaactacgccaactgggtgcaggagaagcccgaccacctgttcaccggcctgatcggcggcaccaacaagcgcgcccccggcgtgcccgcccgcttcagcggcagcctgatcggcgacaaggccgccctgaccatcaccggcgcccagaccgaggacgaggccatctacttctgcgccctgtggtacagcaacctgtgggtgttcggcggcggcaccaagctgaccgtgctg

SEQ ID NO: 69 - protein, 452 aa, synthetic construct
  source 1..452: note = SP34-H PE
EVQLVESGGGLVQPKGSLKLSCAASGFTFNTYAMNWVRQAPGKGLEWVARIRSKYNNYATYYADSVKDRFTISRDDSQSILYLQMNNLKTEDTAMYYCVRHGNFGNSYVSWFAYWGQGTLVTVSSASTKGPSVFPLAPCSRSTSESTAALGCLVKDYFPEPVTVSWNSGALTSGVHTFPAVLQSSGLYSLSSVVTVPSSSLGTKTYTCNVDHKPSNTKVDKRVESKYGPPCPPCPAPEFEGGPSVFLFPPKPKDTLMISRTPEVTCVVVDVSQEDPEVQFNWYVDGVEVHNAKTKPREEQFNSTYRVVSVLTVLHQDWLNGKEYKCKVSNKGLPSSIEKTISKAKGQPREPQVYTLPPSQEEMTKNQVSLTCLVKGFYPSDIAVEWESNGQPENNYKTTPPVLDSDGSFFLYSRLTVDKSRWQEGNVFSCSVMHEALHNHYTQKSLSLSLGK

SEQ ID NO: 70 - DNA, 1356 bp, synthetic construct
  source 1..1356: mol_type = other DNA; note = Nucleotide sequence of SP34-H PE
gaggtgcagctggtggagagcggcggcggcctggtgcagcccaagggcagcctgaagctgagctgcgccgccagcggcttcaccttcaacacctacgccatgaactgggtgcgccaggcccccggcaagggcctggagtgggtggcccgcatccgcagcaagtacaacaactacgccacctactacgccgacagcgtgaaggaccgcttcaccatcagccgcgacgacagccagagcatcctgtacctgcagatgaacaacctgaagaccgaggacaccgccatgtactactgcgtgcgccacggcaacttcggcaacagctacgtgagctggttcgcctactggggccagggcaccctggtgaccgtgagcagcgctagcaccaagggccccagcgtgttccccctggccccctgcagccgcagcaccagcgagagcaccgccgccctgggctgcctggtgaaggactacttccccgagcccgtgaccgtgagctggaacagcggcgccctgaccagcggcgtgcacaccttccccgccgtgctgcagagcagcggcctgtacagcctgagcagcgtggtgaccgtgcccagcagcagcctgggcaccaagacctacacctgcaacgtggaccacaagcccagcaacaccaaggtggacaagcgcgtggagagcaagtacggccctccctgcccaccctgccccgctcccgagtttgaaggcggccccagcgtgttcctgttcccccccaagcccaaggacaccctgatgatcagccgcacccccgaggtgacctgcgtggtggtggacgtgagccaggaggaccccgaggtgcagttcaactggtacgtggacggcgtggaggtgcacaacgccaagaccaagccccgcgaggagcagttcaacagcacctaccgcgtggtgagcgtgctgaccgtgctgcaccaggactggctgaacggcaaggagtacaagtgcaaggtgagcaacaagggcctgcccagcagcatcgagaagaccatcagcaaggccaagggccagccccgcgagccccaggtgtacaccctgccccccagccaggaggagatgaccaagaaccaggtgagcctgacctgcctggtgaagggcttctaccccagcgacatcgccgtggagtgggagagcaacggccagcccgagaacaactacaagaccaccccccccgtgctggacagcgacggcagcttcttcctgtacagcagactgaccgtggacaagagccgctggcaggagggcaacgtgttcagctgcagcgtgatgcacgaggccctgcacaaccactacacccagaagagcctgagcctgagcctgggcaag

SEQ ID NO: 71 - protein, 215 aa, synthetic construct
  source 1..215: note = SP34-L
QAVVTQESALTTSPGETVTLTCRSSTGAVTTSNYANWVQEKPDHLFTGLIGGTNKRAPGVPARFSGSLIGDKAALTITGAQTEDEAIYFCALWYSNLWVFGGGTKLTVLGQPKAAPSVTLFPPSSEELQANKATLVCLISDFYPGAVTVAWKADSSPVKAGVETTTPSKQSNNKYAASSYLSLTPEQWKSHKSYSCQVTHEGSTVEKTVAPTECS

SEQ ID NO: 72 - DNA, 645 bp, synthetic construct
  source 1..645: mol_type = other DNA; note = Nucleotide sequence of SP34-L
caggccgtggtgacccaggagagcgccctgaccaccagccccggcgagaccgtgaccctgacctgccgcagcagcaccggcgccgtgaccaccagcaactacgccaactgggtgcaggagaagcccgaccacctgttcaccggcctgatcggcggcaccaacaagcgcgcccccggcgtgcccgcccgcttcagcggcagcctgatcggcgacaaggccgccctgaccatcaccggcgcccagaccgaggacgaggccatctacttctgcgccctgtggtacagcaacctgtgggtgttcggcggcggcaccaagctgaccgtgctgggtcagcccaaggctgcccctagcgtgacactgttcccaccttctagcgaggaactgcaagcgaataaggctacactggtgtgcctgattagcgacttctaccctggcgccgtgaccgtagcatggaaagcggactctagccccgtgaaggccggcgtggagaccacaaccccatctaagcagtctaacaacaagtacgccgcctcttcctacctgtccctcacccctgagcagtggaagtctcacaagtcttactcttgccaggtgacacacgagggctctacagtggaaaagacagtggcccctacagagtgcagc

SEQ ID NO: 73 - protein, 452 aa, synthetic construct
  source 1..452: note = SP34-H PAA Ks
EVQLVESGGGLVQPKGSLKLSCAASGFTFNTYAMNWVRQAPGKGLEWVARIRSKYNNYATYYADSVKDRFTISRDDSQSILYLQMNNLKTEDTAMYYCVRHGNFGNSYVSWFAYWGQGTLVTVSSASTKGPSVFPLAPCSRSTSESTAALGCLVKDYFPEPVTVSWNSGALTSGVHTFPAVLQSSGLYSLSSVVTVPSSSLGTKTYTCNVDHKPSNTKVDKRVESKYGPPCPPCPAPEAAGGPSVFLFPPKPKDTLMISRTPEVTCVVVDVSQEDPEVQFNWYVDGVEVHNAKTKPREEQFNSTYRVVSVLTVLHQDWLNGKEYKCKVSNKGLPSSIEKTISKAKGQPREPQVYTLPPCQEEMTKNQVSLWCLVKGFYPSDIAVEWESNGQPENNYKTTPPVLDSDGSFFLYSRLTVDKSRWQEGNVFSCSVMHEALHNHYTQKSLSLSLGK

SEQ ID NO: 74 - DNA, 1356 bp, synthetic construct
  source 1..1356: mol_type = other DNA; note = Nucleotide sequence of SP34-H PAA Ks
gaggtgcagctggtggagagcggcggcggcctggtgcagcccaagggcagcctgaagctgagctgcgccgccagcggcttcaccttcaacacctacgccatgaactgggtgcgccaggcccccggcaagggcctggagtgggtggcccgcatccgcagcaagtacaacaactacgccacctactacgccgacagcgtgaaggaccgcttcaccatcagccgcgacgacagccagagcatcctgtacctgcagatgaacaacctgaagaccgaggacaccgccatgtactactgcgtgcgccacggcaacttcggcaacagctacgtgagctggttcgcctactggggccagggcaccctggtgaccgtgagcagcgctagcaccaagggccccagcgtgttccccctggccccctgcagccgcagcaccagcgagagcaccgccgccctgggctgcctggtgaaggactacttccccgagcccgtgaccgtgagctggaacagcggcgccctgaccagcggcgtgcacaccttccccgccgtgctgcagagcagcggcctgtacagcctgagcagcgtggtgaccgtgcccagcagcagcctgggcaccaagacctacacctgcaacgtggaccacaagcccagcaacaccaaggtggacaagcgcgtggagagcaagtacggccccccctgccccccctgccccgcccccgaggccgccggcggccccagcgtgttcctgttcccccccaagcccaaggacaccctgatgatcagccgcacccccgaggtgacctgcgtggtggtggacgtgagccaggaggaccccgaggtgcagttcaactggtacgtggacggcgtggaggtgcacaacgccaagaccaagccccgcgaggagcagttcaacagcacctaccgcgtggtgagcgtgctgaccgtgctgcaccaggactggctgaacggcaaggagtacaagtgcaaggtgagcaacaagggcctgcccagcagcatcgagaagaccatcagcaaggccaagggccagccccgcgagccccaggtgtacaccctgcccccctgccaggaggagatgaccaagaaccaggtgagcctgtggtgcctggtgaagggcttctaccccagcgacatcgccgtggagtgggagagcaacggccagcccgagaacaactacaagaccaccccccccgtgctggacagcgacggcagcttcttcctgtacagcagactgaccgtggacaagagccgctggcaggagggcaacgtgttcagctgcagcgtgatgcacgaggccctgcacaaccactacacccagaagagcctgagcctgagcctgggcaag

SEQ ID NO: 75 - protein, 583 aa, synthetic construct
  source 1..583: note = 05VH-SP34-H PAA
EVQLVESGGGVVQPGRSLRLTCAASGFTFSTSGMYWIRQAPGKGLEWVSYISSSSSTIYYADSVKGRFTISRDNSKNTLYLQMNSLRAEDTAVYYCVTQSCGAGKCYPGVWGQGTTVTVSSGGGGSGGGGSEVQLVESGGGLVQPKGSLKLSCAASGFTFNTYAMNWVRQAPGKGLEWVARIRSKYNNYATYYADSVKDRFTISRDDSQSILYLQMNNLKTEDTAMYYCVRHGNFGNSYVSWFAYWGQGTLVTVSSASTKGPSVFPLAPCSRSTSESTAALGCLVKDYFPEPVTVSWNSGALTSGVHTFPAVLQSSGLYSLSSVVTVPSSSLGTKTYTCNVDHKPSNTKVDKRVESKYGPPCPPCPAPEAAGGPSVFLFPPKPKDTLMISRTPEVTCVVVDVSQEDPEVQFNWYVDGVEVHNAKTKPREEQFNSTYRVVSVLTVLHQDWLNGKEYKCKVSNKGLPSSIEKTISKAKGQPREPQVYTLPPSQEEMTKNQVSLTCLVKGFYPSDIAVEWESNGQPENNYKTTPPVLDSDGSFFLYSRLTVDKSRWQEGNVFSCSVMHEALHNHYTQKSLSLSLGK

SEQ ID NO: 76 - DNA, 1749 bp, synthetic construct
  source 1..1749: mol_type = other DNA; note = Nucleotide sequence of 05VH-SP34-H PAA
gaggtgcagctggtggagtctgggggaggcgtggtccagcctgggaggtccctgagactcacctgtgcagcctctggattcacgttcagtacctctggcatgtactggattcgccaggctccaggcaaggggctggagtgggtttcatacattagtagtagtagtagtaccatatactacgcagactccgtgaagggccggttcaccatctccagagacaattccaagaacacgctgtatctgcaaatgaacagcctgagagctgaggacacggctgtgtattattgtgtgactcagtcgtgtggtgctggtaaatgctacccgggggtctggggccaagggaccacggtcactgtctcctcaggcggaggcggtagcggaggtggagggtctgaggtgcagctggtggagagcggcggcggcctggtgcagcccaagggcagcctgaagctgagctgcgccgccagcggcttcaccttcaacacctacgccatgaactgggtgcgccaggcccccggcaagggcctggagtgggtggcccgcatccgcagcaagtacaacaactacgccacctactacgccgacagcgtgaaggaccgcttcaccatcagccgcgacgacagccagagcatcctgtacctgcagatgaacaacctgaagaccgaggacaccgccatgtactactgcgtgcgccacggcaacttcggcaacagctacgtgagctggttcgcctactggggccagggcaccctggtgaccgtgagcagcgctagcaccaagggccccagcgtgttccccctggccccctgcagccgcagcaccagcgagagcaccgccgccctgggctgcctggtgaaggactacttccccgagcccgtgaccgtgagctggaacagcggcgccctgaccagcggcgtgcacaccttccccgccgtgctgcagagcagcggcctgtacagcctgagcagcgtggtgaccgtgcccagcagcagcctgggcaccaagacctacacctgcaacgtggaccacaagcccagcaacaccaaggtggacaagcgcgtggagagcaagtacggccccccctgccccccctgccccgcccccgaggccgccggcggccccagcgtgttcctgttcccccccaagcccaaggacaccctgatgatcagccgcacccccgaggtgacctgcgtggtggtggacgtgagccaggaggaccccgaggtgcagttcaactggtacgtggacggcgtggaggtgcacaacgccaagaccaagccccgcgaggagcagttcaacagcacctaccgcgtggtgagcgtgctgaccgtgctgcaccaggactggctgaacggcaaggagtacaagtgcaaggtgagcaacaagggcctgcccagcagcatcgagaagaccatcagcaaggccaagggccagccccgcgagccccaggtgtacaccctgccccccagccaggaggagatgaccaagaaccaggtgagcctgacctgcctggtgaagggcttctaccccagcgacatcgccgtggagtgggagagcaacggccagcccgagaacaactacaagaccaccccccccgtgctggacagcgacggcagcttcttcctgtacagcagactgaccgtggacaagagccgctggcaggagggcaacgtgttcagctgcagcgtgatgcacgaggccctgcacaaccactacacccagaagagcctgagcctgagcctgggcaag

SEQ ID NO: 77 - protein, 583 aa, synthetic construct
  source 1..583: note = 05VH-SP34-H PAA Ks
EVQLVESGGGVVQPGRSLRLTCAASGFTFSTSGMYWIRQAPGKGLEWVSYISSSSSTIYYADSVKGRFTISRDNSKNTLYLQMNSLRAEDTAVYYCVTQSCGAGKCYPGVWGQGTTVTVSSGGGGSGGGGSEVQLVESGGGLVQPKGSLKLSCAASGFTFNTYAMNWVRQAPGKGLEWVARIRSKYNNYATYYADSVKDRFTISRDDSQSILYLQMNNLKTEDTAMYYCVRHGNFGNSYVSWFAYWGQGTLVTVSSASTKGPSVFPLAPCSRSTSESTAALGCLVKDYFPEPVTVSWNSGALTSGVHTFPAVLQSSGLYSLSSVVTVPSSSLGTKTYTCNVDHKPSNTKVDKRVESKYGPPCPPCPAPEAAGGPSVFLFPPKPKDTLMISRTPEVTCVVVDVSQEDPEVQFNWYVDGVEVHNAKTKPREEQFNSTYRVVSVLTVLHQDWLNGKEYKCKVSNKGLPSSIEKTISKAKGQPREPQVYTLPPCQEEMTKNQVSLWCLVKGFYPSDIAVEWESNGQPENNYKTTPPVLDSDGSFFLYSRLTVDKSRWQEGNVFSCSVMHEALHNHYTQKSLSLSLGK

SEQ ID NO: 78 - DNA, 1749 bp, synthetic construct
  source 1..1749: mol_type = other DNA; note = Nucleotide sequence of the 05VH-SP34-H PAA Ks
gaggtgcagctggtggagtctgggggaggcgtggtccagcctgggaggtccctgagactcacctgtgcagcctctggattcacgttcagtacctctggcatgtactggattcgccaggctccaggcaaggggctggagtgggtttcatacattagtagtagtagtagtaccatatactacgcagactccgtgaagggccggttcaccatctccagagacaattccaagaacacgctgtatctgcaaatgaacagcctgagagctgaggacacggctgtgtattattgtgtgactcagtcgtgtggtgctggtaaatgctacccgggggtctggggccaagggaccacggtcactgtctcctcaggcggaggcggtagcggaggtggagggtctgaggtgcagctggtggagagcggcggcggcctggtgcagcccaagggcagcctgaagctgagctgcgccgccagcggcttcaccttcaacacctacgccatgaactgggtgcgccaggcccccggcaagggcctggagtgggtggcccgcatccgcagcaagtacaacaactacgccacctactacgccgacagcgtgaaggaccgcttcaccatcagccgcgacgacagccagagcatcctgtacctgcagatgaacaacctgaagaccgaggacaccgccatgtactactgcgtgcgccacggcaacttcggcaacagctacgtgagctggttcgcctactggggccagggcaccctggtgaccgtgagcagcgctagcaccaagggccccagcgtgttccccctggccccctgcagccgcagcaccagcgagagcaccgccgccctgggctgcctggtgaaggactacttccccgagcccgtgaccgtgagctggaacagcggcgccctgaccagcggcgtgcacaccttccccgccgtgctgcagagcagcggcctgtacagcctgagcagcgtggtgaccgtgcccagcagcagcctgggcaccaagacctacacctgcaacgtggaccacaagcccagcaacaccaaggtggacaagcgcgtggagagcaagtacggccccccctgccccccctgccccgcccccgaggccgccggcggccccagcgtgttcctgttcccccccaagcccaaggacaccctgatgatcagccgcacccccgaggtgacctgcgtggtggtggacgtgagccaggaggaccccgaggtgcagttcaactggtacgtggacggcgtggaggtgcacaacgccaagaccaagccccgcgaggagcagttcaacagcacctaccgcgtggtgagcgtgctgaccgtgctgcaccaggactggctgaacggcaaggagtacaagtgcaaggtgagcaacaagggcctgcccagcagcatcgagaagaccatcagcaaggccaagggccagccccgcgagccccaggtgtacaccctgcccccctgccaggaggagatgaccaagaaccaggtgagcctgtggtgcctggtgaagggcttctaccccagcgacatcgccgtggagtgggagagcaacggccagcccgagaacaactacaagaccaccccccccgtgctggacagcgacggcagcttcttcctgtacagcagactgaccgtggacaagagccgctggcaggagggcaacgtgttcagctgcagcgtgatgcacgaggccctgcacaaccactacacccagaagagcctgagcctgagcctgggcaag

SEQ ID NO: 79 - protein, 8 aa, synthetic construct
  source 1..8: note = SP34 H-CDR1
GFTFNTYA

SEQ ID NO: 80 - protein, 10 aa, synthetic construct
  source 1..10: note = SP34 H-CDR2
IRSKYNNYAT

SEQ ID NO: 81 - protein, 16 aa, synthetic construct
  source 1..16: note = SP34 H-CDR3
VRHGNFGNSYVSWFAY

SEQ ID NO: 82 - protein, 9 aa, synthetic construct
  source 1..9: note = SP34 L-CDR1
TGAVTTSNY

SEQ ID NO: 83 - protein, 9 aa, synthetic construct
  source 1..9: note = SP34 L-CDR3
ALWYSNLWV